European Patent Application EP 4 252 907 A1, published October 4, 2023. Title: A methodfor arranging microspheres in a non-aqueous liquid phase. Applicant: Blink AG. The sequence listing filed with the application follows.

SEQUENCE LISTING (3 sequences)

SEQ ID NO: 1 - DNA, 22 bp, Artificial Sequence
  "Forward Primer"
  Forward Primer
ctctgagagcggctctattggt

SEQ ID NO: 2 - DNA, 24 bp, Artificial Sequence
  "Reverse Primer"
  Reverse Primer
gttccctacaacgagcctaaattc

SEQ ID NO: 3 - DNA, 25 bp, Artificial Sequence
  "TaqMan Probe"
  TaqMan Probe
tcagacacgcggtccgctataacga